European Patent Application EP 4 223 305 A1, published August 9, 2023. Title: Drug for preventing or treating fibrotic disease. Applicant: OSAKA UNIVERSITY. The sequence listing filed with the application follows.

SEQUENCE LISTING (21 sequences)

SEQ ID NO: 1 - protein, 7 aa, Homo sapiens
SIKIPSS

SEQ ID NO: 2 - protein, 8 aa, Mus musculus
LMVYVVKT

SEQ ID NO: 3 - protein, 11 aa, Mus musculus
YLQLMVYVVKT

SEQ ID NO: 4 - protein, 8 aa, Homo sapiens
LMVYVTKT

SEQ ID NO: 5 - protein, 11 aa, Homo sapiens
YLQLMVYVTKT

SEQ ID NO: 6 - protein, 9 aa, Mus musculus
HNLMKGGST

SEQ ID NO: 7 - protein, 7 aa, Mus musculus
HNLMKGG

SEQ ID NO: 8 - protein, 9 aa, Homo sapiens
HTLMKGGST

SEQ ID NO: 9 - protein, 7 aa, Homo sapiens
HTLMKGG

SEQ ID NO: 10 - protein, 10 aa, Mus musculus
HETSGSVPAD

SEQ ID NO: 11 - protein, 10 aa, Homo sapiens
HETSGDLATE

SEQ ID NO: 12 - protein, 30 aa, Mus musculus
LMVYVVKTSIKIPSSHNLMKGGSTKNWSGN

SEQ ID NO: 13 - protein, 30 aa, Mus musculus
DYLQLMVYVVKTSIKIPSSHNLMKGGSTKN

SEQ ID NO: 14 - protein, 15 aa, Mus musculus
LMVYVVKTSIKIPSS

SEQ ID NO: 15 - protein, 15 aa, Homo sapiens
LMVYVTKTSIKIPSS

SEQ ID NO: 16 - protein, 22 aa, Mus musculus
LMVYVVKTSIKIPSSHNLMKGG

SEQ ID NO: 17 - protein, 30 aa, Homo sapiens
LMVYVTKTSIKIPSSHTLMKGGSTKYWSGN

SEQ ID NO: 18 - protein, 23 aa, Mus musculus
LMVYVVKTSIKIPSSHNLMKGGS

SEQ ID NO: 19 - protein, 26 aa, Mus musculus
LMVYVVKTSIKIPSSHNLMKGGSTKN

SEQ ID NO: 20 - protein, 24 aa, Mus musculus
LMVYVVKTSIKIPSSHNLMKGGST

SEQ ID NO: 21 - protein, 24 aa, Homo sapiens
LMVYVTKTSIKIPSSHTLMKGGST